European Patent Specification EP 3 497 211 B1, published March 27, 2024. Title: Metabolite Production in Endophytes. Applicant: Agriculture Victoria Services Pty Ltd. The sequence listing filed with the application follows.

SEQUENCE LISTING (28 sequences)

SEQ ID NO: 1 - DNA, 1484 bp, LpTG-3
atgccgtccattccgagtctcgcatcgggcctccaggcatggctcatcagtggcgtcgttctcttgttggcggcggcggcagtgcttgtcggacagatggcggcgtcgcggccgcgccttgacgaccgagcgcctcgtctcctgaagggggcgccgattctcggctgcctcgacttcttccgctgccgaagcgaattcctgctcaaggggagggaccgggaccccagccggcagtttagcttcttctacggaccctatcccattgtcgcattgtctggctctgcggcccggtcctttttctacactgcgcgcggcctcgactttatcccagggtatatcttcaatttaatgctcgtcaaaacgggccgtgggcgagctgacacgctgtgaaatgctagctttctggccctcgttgccgcaggcccgagcatcgagcagctcttacccggcggcgactttcggaccctcttcgtctcgtctttcaagcatttcatgcacaaaaagcagctcgccgccaacctcggttacctgacgaccgacgcagacgtggcccttggcgccatcgacacatcgttgcccgttgagccctttaagctgatgctacacctcatctaccagctcagccaccgcgtcctggggaggcacgacatttccgacgaccccaagctgcttgccgacaccgtgtctgcgtttggactcctcgacgactcgtcggctctcgaggtcatgttcccccgtgtcccctggcccagcaaggtccgcaagatgctcgccggtgccaagttgcaccgcgtgctctccaaaatcacgagcgaccgccgcaagactcgcagaaccaagagggatgccatgcagaccttgatggatcaaggccacccggatactatcgtgtctgccgtacgccctggtccccccgtctcccgctcttatacctcgacacttataccttgcgtacatgtagctcatcatcggcgccctcagtgcaggacttgccaatagcgccttcagtgccgcctggatccttgcctacctttccgtcaaccgcgagtggtacgcccggatacgagccgaagtcgacgctgctgttgccaagcaccgccgctcgcgggtggagtcggcgcccgaagtgctcttgcgcctgtccatgggcgagtgggagtccgagttcccaatgatctgcacggccctacgcgagacgatccgtatgattctgcagctcacgtcaatacgtaaaaatattagcggcaaggatattcagattgccgaaactggcatcatcgcactttgtacttcgtacaaaaataaattaaatataaatatgtgaactaattcaataaatttctttattgatcggactatatcttgatctttttaacttaactatttttaagaattggggggaaggaaagttagctacttagtctttctttcttctttccttaagtttcttaatactatattaacaccctattatagctacctag

SEQ ID NO: 2 - DNA, 1164 bp, LpTG-3
atgccgtccattccgagtctcgcatcgggcctccaggcatggctcatcagtggcgtcgttctcttgttggcggcggcggcagtgcttgtcggacagatggcggcgtcgcggccgcgccttgacgaccgagcgcctcgtctcctgaagggggcgccgattctcggctgcctcgacttcttccgctgccgaagcgaattcctgctcaaggggagggaccgggaccccagccggcagtttagcttcttctacggaccctatcccattgtcgcattgtctggctctgcggcccggtcctttttctacactgcgcgcggcctcgactttatcccaggctttctggccctcgttgccgcaggcccgagcatcgagcagctcttacccggcggcgactttcggaccctcttcgtctcgtctttcaagcatttcatgcacaaaaagcagctcgccgccaacctcggttacctgacgaccgacgcagacgtggcccttggcgccatcgacacatcgttgcccgttgagccctttaagctgatgctacacctcatctaccagctcagccaccgcgtcctggggaggcacgacatttccgacgaccccaagctgcttgccgacaccgtgtctgcgtttggactcctcgacgactcgtcggctctcgaggtcatgttcccccgtgtcccctggcccagcaaggtccgcaagatgctcgccggtgccaagttgcaccgcgtgctctccaaaatcacgagcgaccgccgcaagactcgcagaaccaagagggatgccatgcagaccttgatggatcaaggccacccggatactatcgtgtctgccctcatcatcggcgccctcagtgcaggacttgccaatagcgccttcagtgccgcctggatccttgcctacctttccgtcaaccgcgagtggtacgcccggatacgagccgaagtcgacgctgctgttgccaagcaccgccgctcgcgggtggagtcggcgcccgaagtgctcttgcgcctgtccatgggcgagtgggagtccgagttcccaatgatctgcacggccctacgcgagacgatccgtatgattctgcagctcacgtcaatacgtaaaaatattagcggcaaggatattcagattgccgaaactggcatcatcgcactttctacctag

SEQ ID NO: 3 - protein, 387 aa, LpTG-3
MPSIPSLASGLQAWLISGVVLLLAAAAVLVGQMAASRPRLDDRAPRLLKGAPILGCLDFFRCRSEFLLKGRDRDPSRQFSFFYGPYPIVALSGSAARSFFYTARGLDFIPGFLALVAAGPSIEQLLPGGDFRTLFVSSFKHFMHKKQLAANLGYLTTDADVALGAIDTSLPVEPFKLMLHLIYQLSHRVLGRHDISDDPKLLADTVSAFGLLDDSSALEVMFPRVPWPSKVRKMLAGAKLHRVLSKITSDRRKTRRTKRDAMQTLMDQGHPDTIVSALIIGALSAGLANSAFSAAWILAYLSVNREWYARIRAEVDAAVAKHRRSRVESAPEVLLRLSMGEWESEFPMICTALRETIRMILQLTSIRKNISGKDIQIAETGIIALST

SEQ ID NO: 4 - protein, 377 aa, Hirsutella minnesotensis
SLIPGPEAWPASVLMLLLTGAAAIVIQMVASRPSFPSGAPRLLKGTPILGCLDFFRSRSEFLLKGRDNDPSRQFSFYYGPHPIVVVSGSSARSFFYNARGLDLQAGFSTLFAAGPSLDHLHTGDIRTIFITSFKHLMHKDRLQANLHHLVNDADVALGGLDVSRPVEPFRVMLHLIYQLTHRTLGSNDIAENPKLLAKTLESFGRLDDSSAMEIMFPWVPWPSKMKKMVAGAKLHRTFSNIMNDRRRTGRVEPDAMQTLMDQGHQDLIISIFIIGALFAGLINSAFSAAWILAYLTNNPEWYARIRNEIDAAVAKHRYSEQESAPKVLARLSMDDWETEFPMVDLALRETIRVILQGSSMRKNVSGQDIPIGDTGQI

SEQ ID NO: 5 - DNA, 1844 bp, LpTG-3
cgagcatcaagccgcgtgccgagggaatgtcggacattggccgaaggcgtacatggaccgtatacatcaagccgcaccactgactgcagcctagaaacagatgggcatagttggatatgttgcttcgttattacgtaccgccaatatcctcgatgtgcccctggtgttgctgctctgcagactcgctacggacctcggctggaccgcacccatgctataagccccatcaaggccgatccggttctgcttcatatcctcttgcattaatcccgaagcccgacctttcgtgactgtgctctggcggaacacagatttccggtttgcctactcagcggcaacagttggtaccccgtgacgatccttggagcttgctgccgggataatcatggcatcaacccgggttcttgcgctcccaatgttccccatcttgatgactatttctctttacctcggatactacactcggcggcccattcgccttgtctattgcggcataatattatgcgcctttcttagtgtcgtgcgctgcgcaccacaggacgaggtagggagtgattatgccttcgggatgagtacatacatatccaagcccctaccgtgctgaagagtgttgacgcgtcgagtaaaatagtcggttgcgcgtgcctttgcaaggcattccagatgctcgtcatcgagagagacatctacgccgactattacgagttggatgacaaggaaaagacgcccgtcagatacaggagcctatcgagttgggggaaatgggagtggtgccttgcgcactgcttctctgctcgagggattggctttagctgggccatccctcaccttcccgaggccatgcccagcaacacgacgattcgggactacctgcgggcgagcgctcttaatctcggctggctctaccttgtccaggatctcggacgctcgctgctatctgcggacttgtttgctcacgagggcgtcggagccagcgatacaaagggcggcgcccgttttctgaccgtctattcacttggaatcggggccttgttgaacatcgacatgccataccgtgctgtatgcgccatgggcatggccagcgggtgcttctggaccaggccgcaccacaaccggcctgcagtcggccgctggcgggacgcatggacgctgcgacgcttctggggccgcgtctggcaccagacgttccgcaaggtacgtacatatgcctgcagcggccggccggtgaggagtgctaacgtctgtcccagccctggcagtcgatcggtcaatggattgcctgggaagtcatgcgcgccctcaaaggctcccttgtctcgagatacgtccaggtctacacttcttttctgctatcggccttgatgcacgttgccgctgcgcggatggccgatccgcaccgacgctcctgcgccgggacttggatcttctttctcatgcaggccaacggcatcgtggccgaggatgttgtgcagtgggctggtaagaagacggggatgcgggagtcgtccagcctgacccgtttcctgggccgggcttgggtgctttgctggtttgcatggacggcgccgtggttctttggggatatcgccgacgttggcctgatccgcctcgagacgttccctctgtcggtgactcggggtctgtggaatcggcagtggaagatgtgagacggtgtggaaagtgatgatgatgtattcagctatctaggctatccacacatgtggcacaacgagggcataggtattatcgtgcgctaggcacgtgacttggaaaagatatcccctcgcaggatgataaaggtagaaaaaaggattgaattaaagctatcttctattatataaata

SEQ ID NO: 6 - DNA, 948 bp, LpTG-3
atgctcgtcatcgagagagacatctacgccgactattacgagttggatgacaaggaaaagacgcccgtcagatacaggagcctatcgagttgggggaaatgggagtggtgccttgcgcactgcttctctgctcgagggattggctttagctgggccatccctcaccttcccgaggccatgcccagcaacacgacgattcgggactacctgcgggcgagcgctcttaatctcggctggctctaccttgtccaggatctcggacgctcgctgctatctgcggacttgtttgctcacgagggcgtcggagccagcgatacaaagggcggcgcccgttttctgaccgtctattcacttggaatcggggccttgttgaacatcgacatgccataccgtgctgtatgcgccatgggcatggccagcgggtgcttctggaccaggccgcaccacaaccggcctgcagtcggccgctggcgggacgcatggacgctgcgacgcttctggggccgcgtctggcaccagacgttccgcaagccctggcagtcgatcggtcaatggattgcctgggaagtcatgcgcgccctcaaaggctcccttgtctcgagatacgtccaggtctacacttcttttctgctatcggccttgatgcacgttgccgctgcgcggatggccgatccgcaccgacgctcctgcgccgggacttggatcttctttctcatgcaggccaacggcatcgtggccgaggatgttgtgcagtgggctggtaagaagacggggatgcgggagtcgtccagcctgacccgtttcctgggccgggcttgggtgctttgctggtttgcatggacggcgccgtggttctttggggatatcgccgacgttggcctgatccgcctcgagacgttccctctgtcggtgactcggggtctgtggaatcggcagtggaagatgtga

SEQ ID NO: 7 - protein, 315 aa, LpTG-3
MLVIERDIYADYYELDDKEKTPVRYRSLSSWGKWEWCLAHCFSARGIGFSWAIPHLPEAMPSNTTIRDYLRASALNLGWLYLVQDLGRSLLSADLFAHEGVGASDTKGGARFLTVYSLGIGALLNIDMPYRAVCAMGMASGCFWTRPHHNRPAVGRWRDAWTLRRFWGRVWHQTFRKPWQSIGQWIAWEVMRALKGSLVSRYVQVYTSFLLSALMHVAAARMADPHRRSCAGTWIFFLMQANGIVAEDVVQWAGKKTGMRESSSLTRFLGRAWVLCWFAWTAPWFFGDIADVGLIRLETFPLSVTRGLWNRQWKM

SEQ ID NO: 8 - protein, 391 aa, Oidiodendron maius
MERANFTLLVYLLVPVNLFIASQTPKRFRFLYAVFQLGLYFAIVLLVPPGSVPSSDYTFGTTFYSVLAAFNFFFFCDPYEEHWQIAPEEDKIDQGRDRSRQSSPVKYKDLDLRASVLWCISNAFALRGIGWNWRIPHLPPGPTRGISRVPYLIDVGTTLLKLYLLHDFSATLLEKVTLGGQLPLENIRLDLRTVAVVSFAVSSITLIEFGYQIICFAGAATGLFWTRFQDNHPVIGSVYEGYTIGRFWGRVWHQNMRRAPGKYLAQKVLHVKRGGLVSRYVQSYTAFFLSGVYHYIGAKSSLPHEQLNRTCWFFLLQPNLMLIEDFALWFGKEKLGLKSPRWTCLGYVWTFVMLTVTAAGFVDDCIRHQLVPPTSAFSFSLAALLIQKWEL

SEQ ID NO: 9 - DNA, 1672 bp, LpTG-3
ccgccaccgacataacgagccgttgtctataagagtccaatcgtgccaggacgcaacgtccaagtagccctgattcttgctcaacccgacgtggctcgctttactggcttagagacctcatctgacggccagtctctgattcgaaacccatttgcacgaccgaccaagatgggcacctgttccactcgcgtaggcgagacgccatcgaaaccagcagatgtgacgccgcctgagccatggcaggccctagctcagggtctagggttcgccaatgagaacgagaggtactggtggtccaaacttgcccccctggctggcaagatgatgaagtgggggcagtactcgacgccggagcagtacagagtcctggcattcatacacgcgtatattgtccctagctgtggcccaaggcctggggatggcggtgatctgttctggaaggtgtttctcaactacgattgcacccctatccagctcagtctcaactaccacgatgggaagatgacgcttcggacagctcatatacctatcagcaatatctccggcacagcagaagaccccattaaccagaaggctgcgatagatgccatggtccgccagcaacaggtcctgccgtcccaggacatgcgctggtttaaccactttgtatctaagctcttcctggatcgagatacggcggccaccctcaaggccaaggtggacgagttccagatccggcagggagttcagtgcatgctcagccacgactttcccgacaatcacatccagtgtaagctagcctttgcctcccactggaagtctatcgccactggccttgataaggaggaagttatctgggatgcaatcttggggttaggggacgacgttattccgtataagccagtgctcgctatgctccagcaatactcaacgtccaaaagtgccgcagctgcaggggcacatccgatctttttcgccatcgactcggtgctcaaagacgactatacaagctcacgtatcaagatctattttgttacccaccgaactgcctttaacgtcatggttgacatctataccctaggtggtttgctaatggggccttgtattgaaaagggcacgcaggccttgaggacactctggaaggccgtgctcaatgttcccgaggggtggccagacgataaggatctacccatcaaccccaatggctgtgcggcagtcatcttcaactttgaggtccggcctggcgccgagttcccggctcctaagatttacctcccagcccattactatggccgacccgacttggagattgctgatggaatggaccgctttttcctgagccagggatgggatggtatttaccctggctataagaaaaactacctcaagtgcttgtctgttcttgttgcccctggccttctttccctttgcccttggctaacagtaaggtagtatgaactcggacaaccagctcacggctgtgcaccacgacatttctttttcattcaaggggactaacccctatgttaccgtctattataagcctgagttgcatttggaggctgagtaggcggtggaccaagcggtaaggttagatggggtgttgattccttaattgcttccctttatttttgttattttttgttacgtagcagagttaatggcatctgtcctatgcaggtatttccagggg

SEQ ID NO: 10 - DNA, 1263 bp, LpTG-3
atgggcacctgttccactcgcgtaggcgagacgccatcgaaaccagcagatgtgacgccgcctgagccatggcaggccctagctcagggtctagggttcgccaatgagaacgagaggtactggtggtccaaacttgcccccctggctggcaagatgatgaagtgggggcagtactcgacgccggagcagtacagagtcctggcattcatacacgcgtatattgtccctagctgtggcccaaggcctggggatggcggtgatctgttctggaaggtgtttctcaactacgattgcacccctatccagctcagtctcaactaccacgatgggaagatgacgcttcggacagctcatatacctatcagcaatatctccggcacagcagaagaccccattaaccagaaggctgcgatagatgccatggtccgccagcaacaggtcctgccgtcccaggacatgcgctggtttaaccactttgtatctaagctcttcctggatcgagatacggcggccaccctcaaggccaaggtggacgagttccagatccggcagggagttcagtgcatgctcagccacgactttcccgacaatcacatccagtgtaagctagcctttgcctcccactggaagtctatcgccactggccttgataaggaggaagttatctgggatgcaatcttggggttaggggacgacgttattccgtataagccagtgctcgctatgctccagcaatactcaacgtccaaaagtgccgcagctgcaggggcacatccgatctttttcgccatcgactcggtgctcaaagacgactatacaagctcacgtatcaagatctattttgttacccaccgaactgcctttaacgtcatggttgacatctataccctaggtggtttgctaatggggccttgtattgaaaagggcacgcaggccttgaggacactctggaaggccgtgctcaatgttcccgaggggtggccagacgataaggatctacccatcaaccccaatggctgtgcggcagtcatcttcaactttgaggtccggcctggcgccgagttcccggctcctaagatttacctcccagcccattactatggccgacccgacttggagattgctgatggaatggaccgctttttcctgagccagggatgggatggtatttaccctggctataagaaaaactacctcaagtgcttgtctgttcttgttgcccctggccttctttccctttgcccttggctaacagtaaggtag

SEQ ID NO: 11 - protein, 420 aa, LpTG-3
MGTCSTRVGETPSKPADVTPPEPWQALAQGLGFANENERYWWSKLAPLAGKMMKWGQYSTPEQYRVLAFIHAYIVPSCGPRPGDGGDLFWKVFLNYDCTPIQLSLNYHDGKMTLRTAHIPISNISGTAEDPINQKAAIDAMVRQQQVLPSQDMRWFNHFVSKLFLDRDTAATLKAKVDEFQIRQGVQCMLSHDFPDNHIQCKLAFASHWKSIATGLDKEEVIWDAILGLGDDVIPYKPVLAMLQQYSTSKSAAAAGAHPIFFAIDSVLKDDYTSSRIKIYFVTHRTAFNVMVDIYTLGGLLMGPCIEKGTQALRTLWKAVLNVPEGWPDDKDLPINPNGCAAVIFNFEVRPGAEFPAPKIYLPAHYYGRPDLEIADGMDRFFLSQGWDGIYPGYKKNYLKCLSVLVAPGLLSLCPWLTVR

SEQ ID NO: 12 - protein, 394 aa, Ophiocordyceps unilateralis
MAASPTYENGTPSQPWQALAQGLGYVNQDEQYWWSKVGPLAQRLMEWARYSTPERYRVLAFIYTYIVPACGPKPDDNGQVFWKTYINYDCTPIQLSLNFHDKKVTFRTANISSSDISGTAKDPINQQAAVDAMIKQKRVLPSQNMRWFNHFMSKLFLEPEAAAALKAKADEFQIRNGVQCMLSHDFPNSQVQCKAFFAPNWKAFATGIEMKDVIWDAIMALGDDILPYKSGLAILDRFTTSASAAAAGAVPVCFAFDSVLEGDYKNSRIKIYYATLRTAFDVMVEIYTLGGLLTGPEMEKGVQALRMLWNAVVNIPDGWPDDTDLPANPHRFAAVLFNFEIRHGAELPVPQIYIPAHYYGRSDLEIADGVDRFFQSQGLDADYPPYKENYIKCL

SEQ ID NO: 13 - DNA, 1992 bp, LpTG-3
tcctgaccatgttggctccgccaacggtgagactcacccttgttctgacacgcataccgcgagagtaatatttcatgtacatgaacaaagcgcacggtgcggtatcttgcgtttaattattgctccatattgcaggctgcatatgcattacgggagatggttgcattcaatgccatatgatgccgaggagagcggccgatacgcgccccgcctgtgctgtcccggattgaagaaatgcccgaggaaatgggatctgttggctataatagcaagggaagtaagcgtgtatcatccccggaaccatcaagcactaccgctttgaatcgcttctcttcttgacagcatgggagaccctcttcccggcaacacgcgagactgtctctcccgcaacatgcgagactcctcaaccgagaagctccccattctgtggcggaccgactcccccctcaaccagtacgatgaagcacggtgcagagtcttcaacggcaggcggcccgagcatttcccacgcgcaatcgtccaggccacgacgctcgaccacatcgtagcggctgtgaggctggccgtggagtccgccgcccctgtggccgtccgctcaggtggccacagtctctcctgctggaccatgcgccatgatgccatcctcattgatctcaaggactttagctatctaagctacgatgaagaaacacaccaagtccaggcctctcccagtaccctaacgggagaattgctcgagtttcttgcccagaagcagcgattctttcccgtaggccactcagggggcattggcctaggtggctacctcctccaagctggaatcggactcaactgccgggtatgcgtgcttgctctgcctgccccatgcttgcctatccgtttctcttcatccactgacggcaacgtctagggctatgggtacgcatgcgagtctgtctctggaatcgacattgttaccgccgatggctgcattaagcactgtgacaaagaagaaaacgctgatttgtattgggccgctcgcggagctgggccgggtgagtccctctctgaaagccttccgcattaaagccgtggcaaatctaactaaacagagttccctgccattgtcacacgcttctacctcgagactcgaccgatgccggtttgcaaccggagcacgtacatctggccggcgaccatgtatgaccaggttttcccttggctcgaccgcgtgagtagctcgtgtccatgtccccagccaagctcacgaggtttcaagctcttaactacgctggacgagaacgtcgaggttggcgtgttcggatttacagtcccccaactcaaccagccggggctacacgtgctcgcaacagcattcggagactcggatgaggatacccggcgaatgctcacacccttcatcgacacccaccccccaggagcgattcacgcccaggactttgtggcgactgacttcgctagcgactacgttctagataagacagtcctgccgcaaggtgctcgttacttcaccgatagcgtctttctcaagcctggcaccgacctagtggtggcttgtaaggacatgtttacaggactaaagcatccgcgcgcattggcatattggcagccgatgaagaccgccactgcccgcacccttcccgacatggccatgagcatacatagcgaccattacgtatccctactaggaatctacgacgattccgcccaagacgatgagcagacgtcctggatcgtggattatatgcgtaagctggagccatttgtcttgggcacgtttgtgggggatgcgcatgtgttggaaagaccgtctaattactggtcagaggaggccaaagagcgagtgctccgtgttggaaagaagtgggatcctagtggaagaattcgggggatgctcctcagtgactcgtaggcagcgatttatttaaagggcgtgcttatcaggcaaacgcgtacgcgtaattagcacccctaaaggtagctaaggtagct

SEQ ID NO: 14 - DNA, 1440 bp, LpTG-3
atgggagaccctcttcccggcaacacgcgagactgtctctcccgcaacatgcgagactcctcaaccgagaagctccccattctgtggcggaccgactcccccctcaaccagtacgatgaagcacggtgcagagtcttcaacggcaggcggcccgagcatttcccacgcgcaatcgtccaggccacgacgctcgaccacatcgtagcggctgtgaggctggccgtggagtccgccgcccctgtggccgtccgctcaggtggccacagtctctcctgctggaccatgcgccatgatgccatcctcattgatctcaaggactttagctatctaagctacgatgaagaaacacaccaagtccaggcctctcccagtaccctaacgggagaattgctcgagtttcttgcccagaagcagcgattctttcccgtaggccactcagggggcattggcctaggtggctacctcctccaagctggaatcggactcaactgccggggctatgggtacgcatgcgagtctgtctctggaatcgacattgttaccgccgatggctgcattaagcactgtgacaaagaagaaaacgctgatttgtattgggccgctcgcggagctgggccggagttccctgccattgtcacacgcttctacctcgagactcgaccgatgccggtttgcaaccggagcacgtacatctggccggcgaccatgtatgaccaggttttcccttggctcgaccgcgtgagtagctcgtgtccatgtccccagccaagctcacgaggtttcaagctcttaactacgctggacgagaacgtcgaggttggcgtgttcggatttacagtcccccaactcaaccagccggggctacacgtgctcgcaacagcattcggagactcggatgaggatacccggcgaatgctcacacccttcatcgacacccaccccccaggagcgattcacgcccaggactttgtggcgactgacttcgctagcgactacgttctagataagacagtcctgccgcaaggtgctcgttacttcaccgatagcgtctttctcaagcctggcaccgacctagtggtggcttgtaaggacatgtttacaggactaaagcatccgcgcgcattggcatattggcagccgatgaagaccgccactgcccgcacccttcccgacatggccatgagcatacatagcgaccattacgtatccctactaggaatctacgacgattccgcccaagacgatgagcagacgtcctggatcgtggattatatgcgtaagctggagccatttgtcttgggcacgtttgtgggggatgcgcatgtgttggaaagaccgtctaattactggtcagaggaggccaaagagcgagtgctccgtgttggaaagaagtgggatcctagtggaagaattcgggggatgctcctcagtgactcgtag

SEQ ID NO: 15 - protein, 479 aa, LpTG-3
MGDPLPGNTRDCLSRNMRDSSTEKLPILWRTDSPLNQYDEARCRVFNGRRPEHFPRAIVQATTLDHIVAAVRLAVESAAPVAVRSGGHSLSCWTMRHDAILIDLKDFSYLSYDEETHQVQASPSTLTGELLEFLAQKQRFFPVGHSGGIGLGGYLLQAGIGLNCRGYGYACESVSGIDIVTADGCIKHCDKEENADLYWAARGAGPEFPAIVTRFYLETRPMPVCNRSTYIWPATMYDQVFPWLDRVSSSCPCPQPSSRGFKLLTTLDENVEVGVFGFTVPQLNQPGLHVLATAFGDSDEDTRRMLTPFIDTHPPGAIHAQDFVATDFASDYVLDKTVLPQGARYFTDSVFLKPGTDLVVACKDMFTGLKHPRALAYWQPMKTATARTLPDMAMSIHSDHYVSLLGIYDDSAQDDEQTSWIVDYMRKLEPFVLGTFVGDAHVLERPSNYWSEEAKERVLRVGKKWDPSGRIRGMLLSDS

SEQ ID NO: 16 - protein, 444 aa, Escovopsis weberi
MADLPIIWRSDTESAAKYEEARCRIFNIRRPEHFPRAIVKATTLEHIVAAVKLAAEQGVRVVARSGGHGLSAWTLRHNAILIDLQNFKHMSYDEEKNEAQVSPSTLAEELLDFLAERKRFFPAGHTGDIGLGGYLLQGGIGLSCRGYGYACEYVTGVDVVTAEGDVVHADENENADLYWAARGAGPEFPAIVTRFYLKTIPLQPVAKGCRYIWPAVMYDAIFSWIDKISASLDEHVDPSVFGFMIPGINQPGLMFSASVFAQTEEEARRKLAPLVETHPPGAMVAEDFVDSSITTVYAGSRQFNPPGCRYFTDSVFLKPGTDVVEACRHMFTQIPFPRGLAYWQPLRISPARKQPDMALSIQSEHYVSLLAVYDNEAEDEAQTEWVIEGIRKLEPQIHGTFIADAHPEMRTSNYWSEEATARLAAVGSKWDPKGRITGIVVRQE

SEQ ID NO: 17 - DNA, 1263 bp, LpTG-3
ctaccttactgttagccaagggcaaagggaaagaaggccaggggcaacaagaacagacaagcacttgaggtagtttttcttatagccagggtaaataccatcccatccctggctcaggaaaaagcggtccattccatcagcaatctccaagtcgggtcggccatagtaatgggctgggaggtaaatcttaggagccgggaactcggcgccaggccggacctcaaagttgaagatgactgccgcacagccattggggttgatgggtagatccttatcgtctggccacccctcgggaacattgagcacggccttccagagtgtcctcaaggcctgcgtgcccttttcaatacaaggccccattagcaaaccacctagggtatagatgtcaaccatgacgttaaaggcagttcggtgggtaacaaaatagatcttgatacgtgagcttgtatagtcgtctttgagcaccgagtcgatggcgaaaaagatcggatgtgcccctgcagctgcggcacttttggacgttgagtattgctggagcatagcgagcactggcttatacggaataacgtcgtcccctaaccccaagattgcatcccagataacttcctccttatcaaggccagtggcgatagacttccagtgggaggcaaaggctagcttacactggatgtgattgtcgggaaagtcgtggctgagcatgcactgaactccctgccggatctggaactcgtccaccttggccttgagggtggccgccgtatctcgatccaggaagagcttagatacaaagtggttaaaccagcgcatgtcctgggacggcaggacctgttgctggcggaccatggcatctatcgcagccttctggttaatggggtcttctgctgtgccggagatattgctgataggtatatgagctgtccgaagcgtcatcttcccatcgtggtagttgagactgagctggataggggtgcaatcgtagttgagaaacaccttccagaacagatcaccgccatccccaggccttgggccacagctagggacaatatacgcgtgtatgaatgccaggactctgtactgctccggcgtcgagtactgcccccacttcatcatcttgccagccaggggggcaagtttggaccaccagtacctctcgttctcattggcgaaccctagaccctgagctagggcctgccatggctcaggcggcgtcacatctgctggtttcgatggcgtctcgcctacgcgagtggaacaggtgcccat

SEQ ID NO: 18 - DNA, 129 bp, LpTG-3
gcggtccattccatcagcaatctccaagtcgggtcggccatagtaatgggctgggaggtaaatcttaggagccgggaactcggcgccaggccggacctcaaagttgaagatgactgccgcacagccatt

SEQ ID NO: 19 - DNA, 95 bp, LpTG-3
cccaagattgcatcccagataacttcctccttatcaaggccagtggcgatagacttccagtgggaggcaaaggctagcttacactggatgtgatt

SEQ ID NO: 20 - DNA, 561 bp, LpTG-3
gcggtccattccatcagcaatctccaagtcgggtcggccatagtaatgggctgggaggtaaatcttaggagccgggaactcggcgccaggccggacctcaaagttgaagatgactgccgcacagccattccaagattgcatcccagataacttcctccttatcaaggccagtggcgatagacttccagtgggaggcaaaggctagcttacactggatgtgattgtcgggaaagtcgtggctgagcatgcactgaactccctgccggatctggaactcgtccaccttggccttgagggtggccgccgtatctcgatccaggaagagcttagatacaaagtggttaaaccagcgcatgtcctgggacggcaggacctgttgctggcggaccatggcatctatcgcagccttctggttaatggggtcttctgctgtgccggagatattgctgataggtatatgagctgtccgaagcgtcatcttcccatcgtggtagttgagactgagctggataggggtgcaatcgtagttgagaaacaccttccagaacagatcaccgccat

SEQ ID NO: 21 - DNA, 20 bp, Artificial Sequence
  Primer
tgtcgtccatcacagtttgc

SEQ ID NO: 22 - DNA, 20 bp, Artificial Sequence
  Primer
gcgccgatggtttctacaaa

SEQ ID NO: 23 - DNA, 20 bp, Artificial Sequence
  Primer
gcctttcttcttgcctgtca

SEQ ID NO: 24 - DNA, 20 bp, Artificial Sequence
  Primer
gaccgcctgtgtgttttgaa

SEQ ID NO: 25 - DNA, 20 bp, Artificial Sequence
  Primer
cacacagcccaagattgcat

SEQ ID NO: 26 - DNA, 20 bp, Artificial Sequence
  Primer
tggaagtctatcgccactgg

SEQ ID NO: 27 - DNA, 20 bp, Artificial Sequence
  Primer
ggagttcagtgcatgctcag

SEQ ID NO: 28 - DNA, 20 bp, Artificial Sequence
  Primer
ggcaagaagaaaggctcacc